European Patent Application EP 4 177 344 A1, published May 10, 2023. Title: A Novel Cell for Transplantation with Reduced Immunogenicity. Applicant: GREEN CROSS LABCELL. The sequence listing filed with the application follows.

SEQUENCE LISTING (46 sequences)

SEQ ID NO: 1 - RNA, 20 nt, Artificial Sequence
  B2M-gRNA -1
atccatccgacattgaagtt

SEQ ID NO: 2 - RNA, 21 nt, Artificial Sequence
  B2M-gRNA -2
atccatccgacattgaagttg

SEQ ID NO: 3 - RNA, 23 nt, Artificial Sequence
  B2M-gRNA-3
atccatccgacattgaagttgac

SEQ ID NO: 4 - RNA, 22 nt, Artificial Sequence
  B2M-gRNA-4
ttagagtctcgtgatgtttaag

SEQ ID NO: 5 - RNA, 22 nt, Artificial Sequence
  B2M-gRNA-5
ccgauauuccucagguacucca

SEQ ID NO: 6 - RNA, 21 nt, Artificial Sequence
  B2M-gRNA-6
atataagtggaggcgtcgcgc

SEQ ID NO: 7 - RNA, 23 nt, Artificial Sequence
  B2M-gRNA-7
atataagtggaggcgtcgcgctg

SEQ ID NO: 8 - RNA, 21 nt, Artificial Sequence
  B2M-gRNA-8
agtgggggtgaattcagtgta

SEQ ID NO: 9 - RNA, 23 nt, Artificial Sequence
  B2M-gRNA-9
agtgggggtgaattcagtgtagt

SEQ ID NO: 10 - RNA, 21 nt, Artificial Sequence
  B2M-gRNA-10
ctgaattgctatgtgtctggg

SEQ ID NO: 11 - RNA, 23 nt, Artificial Sequence
  B2M-gRNA-11
ctgaattgctatgtgtctgggtt

SEQ ID NO: 12 - RNA, 21 nt, Artificial Sequence
  B2M-gRNA-12
ctcacgtcatccagcagagaa

SEQ ID NO: 13 - RNA, 23 nt, Artificial Sequence
  B2M-gRNA-13
ctcacgtcatccagcagagaatg

SEQ ID NO: 14 - RNA, 21 nt, Artificial Sequence
  B2M-gRNA-14
agcaaggactggtctttctat

SEQ ID NO: 15 - RNA, 23 nt, Artificial Sequence
  B2M-gRNA-15
agcaaggactggtctttctatct

SEQ ID NO: 16 - RNA, 23 nt, Artificial Sequence
  B2M-gRNA-16
cattctctgctggatgacgtgag

SEQ ID NO: 17 - RNA, 23 nt, Artificial Sequence
  B2M-gRNA-17
tcagtgggggtgaattcagtgta

SEQ ID NO: 18 - RNA, 23 nt, Artificial Sequence
  B2M-gRNA-18
cagtgggggtgaattcagtgtag

SEQ ID NO: 19 - RNA, 23 nt, Artificial Sequence
  B2M-gRNA-19
tcacagcccaagatagttaagtg

SEQ ID NO: 20 - RNA, 23 nt, Artificial Sequence
  CIITA-gRNA-1
ccttggggctctgacaggtagga

SEQ ID NO: 21 - RNA, 23 nt, Artificial Sequence
  CIITA-gRNA-2
ccggcctttttaccttggggctc

SEQ ID NO: 22 - RNA, 23 nt, Artificial Sequence
  CIITA-gRNA-3
ctcccagaacccgacacagacac

SEQ ID NO: 23 - RNA, 23 nt, Artificial Sequence
  CIITA-gRNA-4
cttgtctgggcagcggaactgga

SEQ ID NO: 24 - RNA, 23 nt, Artificial Sequence
  CIITA-gRNA-5
tgcccaacttctgctggcatctc

SEQ ID NO: 25 - RNA, 23 nt, Artificial Sequence
  CIITA-gRNA-6
tgacttttctgcccaacttctgc

SEQ ID NO: 26 - RNA, 23 nt, Artificial Sequence
  CIITA-gRNA-7
tccaggcgcatctggccggaggc

SEQ ID NO: 27 - RNA, 23 nt, Artificial Sequence
  CIITA-gRNA-8
tccccaccatctccactctgccc

SEQ ID NO: 28 - RNA, 23 nt, Artificial Sequence
  CIITA-gRNA-9
tccagttcctcgttgagctgcct

SEQ ID NO: 29 - RNA, 23 nt, Artificial Sequence
  CIITA-gRNA-10
ccagagcccatggggcagagtgg

SEQ ID NO: 30 - RNA, 23 nt, Artificial Sequence
  CIITA-gRNA-11
ctcgggaggtcagggcaggttca

SEQ ID NO: 31 - RNA, 23 nt, Artificial Sequence
  CIITA-gRNA-12
gaagcttgttggagacctctcca

SEQ ID NO: 32 - RNA, 23 nt, Artificial Sequence
  CIITA-gRNA-13
gcagcacgtggtacaggagctcc

SEQ ID NO: 33 - RNA, 23 nt, Artificial Sequence
  CIITA-gRNA-14
gccatcgcccaggtcctcacgtc

SEQ ID NO: 34 - RNA, 23 nt, Artificial Sequence
  CIITA-gRNA-15
agagctcagggatgacagagcac

SEQ ID NO: 35 - RNA, 23 nt, Artificial Sequence
  CIITA-gRNA-16
cagtaggagtagtcgtcgcgtat

SEQ ID NO: 36 - RNA, 23 nt, Artificial Sequence
  CIITA-gRNA-17
cagggcaagggtgcgcaggcgca

SEQ ID NO: 37 - RNA, 23 nt, Artificial Sequence
  CIITA-gRNA-18
cgagatctactgaaccagaaaag

SEQ ID NO: 38 - RNA, 23 nt, Artificial Sequence
  CIITA-gRNA-19
tggttcagtagatctcgtaaaga

SEQ ID NO: 39 - RNA, 23 nt, Artificial Sequence
  CIITA-gRNA-20
ggacaaggttctctgcaacctga

SEQ ID NO: 40 - RNA, 21 nt, Artificial Sequence
  CIITA-gRNA-21
ccttggggctctgacaggtag

SEQ ID NO: 41 - RNA, 21 nt, Artificial Sequence
  CIITA-gRNA-22
gggctctgacaggtaggaccc

SEQ ID NO: 42 - RNA, 21 nt, Artificial Sequence
  CIITA-gRNA-23
cctcccaggcagctcacagtg

SEQ ID NO: 43 - RNA, 21 nt, Artificial Sequence
  CIITA-gRNA-24
tatgaccagatggacctggct

SEQ ID NO: 44 - RNA, 21 nt, Artificial Sequence
  CIITA-gRNA-25
tgcccaacttctgctggcatc

SEQ ID NO: 45 - protein, 33 aa, Artificial Sequence
  FSD64d1
LLKIWSRLIKIWTQGRRLGGSGGGSARAARQAR

SEQ ID NO: 46 - DNA, 1503 bp, Artificial Sequence
  codon-optimized HLA-E
atgtctcgctccgtggctctggctgtcctggctctgctgagtctgtctgggctggaagctgtgatggcaccaagaaccctgatcctgggaggaggaggatccggaggaggaggatctggcggcggcggcagcatccagcgcacccctaagatccaggtgtatagccggcacccagccgagaacggcaagtccaacttcctgaattgctacgtgtccggctttcacccatctgacatcgaggtggatctgctgaagaatggcgagagaatcgagaaggtggagcactctgacctgtctttcagcaaggattggagcttttatctgctgtactataccgagttcacccctacagagaaggacgagtacgcctgtcgcgtgaaccacgtgacactgagccagccaaagatcgtgaagtgggaccgggatatgggaggaggaggaagcggaggaggaggaagcggcggcggcggctctggcggcggcggctccggctctcacagcctgaagtatttccacacctccgtgtctaggccaggaaggggagagccacggttcatcagcgtgggctacgtggacgatacacagttcgtgaggtttgacaatgatgcagcctccccaagaatggtgcctagggcaccatggatggagcaggagggatccgagtactgggaccgggagacaagatctgccagggatacagcccagatctttcgcgtgaacctgcgcaccctgaggggatactataatcagtctgaggccggcagccacacactgcagtggatgcacggatgcgagctgggacctgatcggagattcctgcgcggctacgagcagtttgcctatgacggcaaggattacctgaccctgaacgaggacctgcggagctggaccgcagtggatacagcagcccagatctccgagcagaagtctaatgacgccagcgaggcagagcaccagagggcatatctggaggatacctgcgtggagtggctgcacaagtacctggagaagggcaaggagacactgctgcacctggagccccctaagacccacgtgacacaccacccaatctccgaccacgaggccaccctgagatgttgggccctgggcttctatcccgccgagatcaccctgacatggcagcaggacggagagggacacacccaggatacagagctggtggagacacggcccgcaggcgatggcacatttcagaagtgggcagcagtggtggtgccttctggagaggagcagagatacacatgtcacgtgcagcacgagggcctgccagagccagtgaccctgaggtggaagcctgcctcccagcccacaatccctatcgtgggaatcatcgcaggcctggtgctgctgggcagcgtggtgtccggagcagtggtggcagccgtgatctggaggaagaagagctccggcggcaagggcgggtcctactacaaagcagaatggtccgactccgcacaggggtccgagagccactcactgtaa